European Patent Specification EP 2 906 682 B1, published June 11, 2025. Title: BACTERIAL LIVE VECTOR VACCINES EXPRESSING CHROMOSOMALLY-INTEGRATED FOREIGN ANTIGENS. Applicant: Galen, James E Wang, Jin-Yuang. The sequence listing filed with the application follows.

SEQUENCE LISTING (44 sequences)

SEQ ID NO: 1 - DNA, 29 bp, Artificial Sequence
  Primer 5guaBA-for
gaattctagctgctcatacttctgctgca

SEQ ID NO: 2 - DNA, 30 bp, Artificial Sequence
  Primer 5guaBA-rev
gctagccaattggggcaatatctcacctgg

SEQ ID NO: 3 - DNA, 32 bp, Artificial Sequence
  Primer 3guaBA-for
ggatccactagtgtcgataacccttcctgtgt

SEQ ID NO: 4 - DNA, 29 bp, Artificial Sequence
  Primer 3guaBA-rev
ctcgagacagcacctacaagtctggcatg

SEQ ID NO: 5 - DNA, 24 bp, Artificial Sequence
  Primer guaBA PCR-for
gcgctgaccaccggaatacggctg

SEQ ID NO: 6 - DNA, 28 bp, Artificial Sequence
  Primer guaBA PCR-rev
catggcatggatgaggcaaccgcgaagc

SEQ ID NO: 7 - DNA, 36 bp, Artificial Sequence
  Primer 5htrA-for
gaattcgtaccttcaatcaggcgttactggaagatg

SEQ ID NO: 8 - DNA, 49 bp, Artificial Sequence
  Primer 5htrA-rev
gctagccaattgcgattaacaggtaacgcaaaattgctgtgtacgtcag

SEQ ID NO: 9 - DNA, 44 bp, Artificial Sequence
  Primer 3htrA-for
ggatccactagtctgcgtaagattctcgacagcaagccgtcggt

SEQ ID NO: 10 - DNA, 42 bp, Artificial Sequence
  Primer 3htrA-rev
ctcgagccagcatcatttcggcagtcatacacaccagttcgc

SEQ ID NO: 11 - DNA, 29 bp, Artificial Sequence
  Primer htrA PCR-for
gtgtcgccgatcttgaagacgcggtagag

SEQ ID NO: 12 - DNA, 29 bp, Artificial Sequence
  Primer htrA PCR-rev
ctatcgacgccaagctggccgctgtcgac

SEQ ID NO: 13 - DNA, 51 bp, Artificial Sequence
  Primer 5clyA-for
tagtaatgagaattcgctggtattgatcggctctccggtagagattagcga

SEQ ID NO: 14 - DNA, 49 bp, Artificial Sequence
  Primer 5clyA-rev
gctagccaattgtgcctctttaaatatataaattgcaattaagtacctg

SEQ ID NO: 15 - DNA, 56 bp, Artificial Sequence
  Primer 3clyA-for
ggatccactagtgatacattttcattcgatctgtgtacttttaacgcccgatagcg

SEQ ID NO: 16 - DNA, 57 bp, Artificial Sequence
  Primer 3clyA-rev
tgatagtaactcgagacaatccataagaaaggtcaggcacactgggaaggcgacatc

SEQ ID NO: 17 - DNA, 27 bp, Artificial Sequence
  Primer clyA PCR-for
catgatggtatccagtatggcacaagc

SEQ ID NO: 18 - DNA, 27 bp, Artificial Sequence
  Primer clyA PCR-rev
gtaatcgacaacatgctacatccatcg

SEQ ID NO: 19 - DNA, 33 bp, Artificial Sequence
  Primer 5FRT-aph-for
gaattcgctagcgctggagctgcttcgaagttc

SEQ ID NO: 20 - DNA, 33 bp, Artificial Sequence
  Primer 3FRT-aph-rev
ctcgagttccggggatccgtcgacctgcagttc

SEQ ID NO: 21 - DNA, 32 bp, Artificial Sequence
  Primer 5gfpuv
caattgtgtggtagcacagaataatgaaaagt

SEQ ID NO: 22 - DNA, 30 bp, Artificial Sequence
  Primer 3gfpuv
gctagctcattatttgtagagctcatccat

SEQ ID NO: 23 - DNA, 996 bp, Artificial Sequence
  codon-optimized gene cassette tcdA-14CBD/A
tagtaatgaatggctagcaccggctatacgagcatcaacgggaagcatttttatttcaataccgacggcattatgcagatcggggtgttcaaagggcccaacggtttcgaatactttgcgccggccaacacggatgcgaataacatcgaaggtcaagccatcctctaccagaacaaattcctgaccctcaatggcaagaaatattacttcgggtccgacagcaaggctgtcacgggtctgcgcacgattgatgggaaaaagtattacttcaacaccaatactgccgtggcggtcaccggatggcaaacgatcaacggcaagaaatactacttcaataccaacacgtccattgcctcgaccgggtatacgatcatttccggcaaacacttctacttcaacaccgacgggatcatgcaaatcggtgtgtttaaagggcccgatggcttcgagtactttgccccggcgaatacggacgccaataacattgaaggtcaggcaattcggtatcagaatcgttttctctatctgcatgacaacatctactatttcggtaataacagcaaggcggccaccgggtgggtcacgattgatggcaaccggtattacttcgagcccaatacggcgatgggggcgaatggttataaaacgatcgacaacaagaatttctactttcgcaacgggctcccgcagattggcgtgttcaaagggtccaacggctttgagtacttcgcccccgcgaatacggatgccaacaatatcgagggccaagcgattcggtatcaaaaccgcttcctccacctgctcgggaaaatctattacttcggcaataactcgaaagccgtcacgggttggcaaacgattaatggcaaagtgtattacttcatgccggatactgcaatggcagccgctggtggattattcgaaattgacggcgtcatctatttctttggcgtggatggggtcaaagccccggggatctatggctaatgacctagg

SEQ ID NO: 24 - DNA, 1629 bp, Artificial Sequence
  codon-optimized gene cassette TcdB CBD/B
tagtaatgaatggctagcggcctgatctatattaacgattcactgtactatttcaagccgcccgtcaataacctcatcaccgggtttgtgacggtcggcgacgataaatactacttcaatccgatcaacggcggagccgcgagcattggggagaccatcattgatgacaagaattattacttcaaccagagtggcgtgctgcagacgggggtcttcagtaccgaggacggctttaaatacttcgcccccgcgaatacgctcgatgagaacctggaaggggaggcgattgactttaccggcaagctgatcattgacgagaacatctactatttcgatgacaattaccgcggggccgtggaatggaaggagctcgatggcgagatgcactattttagcccggagacggggaaagctttcaaaggcctgaatcaaattggggactacaagtattacttcaactctgacggtgtgatgcagaaggggttcgtgagtatcaatgacaacaagcattatttcgacgattctggcgtcatgaaagtggggtacaccgagatcgatggcaagcacttctactttgccgagaatggtgagatgcaaatcggcgtgttcaatacggaagacgggtttaagtatttcgcgcatcataacgaggatctcggcaatgaagagggcgaagagatctcatattccggaatcctcaacttcaataacaagatttactactttgatgactcatttaccgccgtggtcggctggaaggacctcgaggatgggtcaaagtactatttcgacgaggatacggcggaggcctacatcggcctgtcattaatcaacgacggccagtattactttaatgatgacggcatcatgcaggtcgggtttgtcaccatcaacgataaagtcttctacttctctgactctggcattatcgagagcggggtgcagaacatcgacgataactatttctacatcgatgacaatggcattgtccagatcggcgtgttcgatacgtcagacggttataagtattttgcgcccgccaacaccgtcaacgataatatctacggtcaagctgttgaatatagtggtttggtccgtgtcggtgaagacgtgtactatttcggcgagacgtacacaattgagacgggctggatctatgatatggagaacgagagtgacaagtactatttcaatcctgagaccaagaaagcatgcaaggggatcaacctgatcgatgacatcaagtactatttcgacgagaagggcattatgcgcacggggcttatctcatttgagaataacaattattacttcaatgagaacggggaaatgcagtttgggtacatcaatattgaggacaagatgttctattttggcgaggatggcgtcatgcagatcggggtgttcaacaccccagatggtttcaagtatttcgcgcatcagaatacgctggatgagaacttcgagggcgaatcaatcaactataccgggtggctggacctcgatgagaagcgctactatttcacggacgaatacattgcggccaccggctcagtcatcattgatggcgaggaatactatttcgaccctgatacggcgcagctggtgatcagtgagtaatgacctagg

SEQ ID NO: 25 - DNA, 43 bp, Artificial Sequence
  Primer 5rpoS-for
aagcttgaattccgtattctgagggctcaggtgaacaaagtgc

SEQ ID NO: 26 - DNA, 43 bp, Artificial Sequence
  Primer 5rpoS-rev
cctaggcaattgacccgtgatcccttgacggaactagcaagtc

SEQ ID NO: 27 - DNA, 39 bp, Artificial Sequence
  Primer 3rpoS-for
ggatccggttcggtatcgcgccaggtatacagacaatgc

SEQ ID NO: 28 - DNA, 38 bp, Artificial Sequence
  Primer 3rpoS-rev
ctcgagccggaagtgcaggcggtaaacgctatgtacac

SEQ ID NO: 29 - DNA, 27 bp, Artificial Sequence
  Primer rpoS PCR-for
atgcagcacagcaaggagttgtgacca

SEQ ID NO: 30 - DNA, 31 bp, Artificial Sequence
  Primer rpoS PCR-rev
ggtgcgtatcgataaggtctcttaccacagc

SEQ ID NO: 31 - DNA, 3290 bp, Artificial Sequence
  5guaB-PompC-14CBDA-FRT-3guaA gene cassette
gcgctgaccaccggaatacggctggcaaaaatagcccgcgccacgcgttcgtcgttaaaactccacaaatcttccagcgaaccgccgccgcgtccgacgatcagcacgtcgcactcgccgcgcgtgtttgccagttcgatagcacgaacgatctgccccggcgcatcgtcgccctgtaccgcggttggatagataataacgggcagggatgggtcacgacgcttcaacacgtggaggatatcgtgcagcgccgcgccggttttcgaggtgatcaccccaacgcagtgggccggggagggcaacggctgtttatgctgctgatcgaacaagccttcggcatggagtttggcttttagctgctcatacttctgctgcaacaagccttcgccagccggctgcatactttcggcgatgatttgataatcgccgcgcggctcgtacagcgtaatgttggcgcgtaccagcacctgctgcccgtgctgcgggcggaacgtcacccggcggttgctgttgcggaacatcgcacagcgcacctgagcggtatcgtctttgagcgtaaagtaccagtggcccgacgcaggctgcgtgaaattagaaatctcgccgctgatccatacctgtcccatctcctgttctaacagcagacgaaccgtctggttaaggcggcttacggtaaaaattgaggaagtttgagaggataacatgtgagcgggatcaaattctaaatcagcaggttattcaatcgatagtaacctgctcacgggggatcgcaagcactatttgcaaaaaaatgtagatgcaaccgattacgttctgtataatgccgcggcaatatttattaacctcccaggtgagatattgccccaattcgtcaattctgtggtagcacagaataatgaaaagtgtgtaaagaagggtaaaaaaaaccgaatgcgaggcatccggttgaaataggggtaaacagacattcagaaatgaatgacggtaataaataaagttaatgatgatagcgggagttattctagttgcgagtgaaggttttgttttgacattcagtgctgtcaaatacttaagaataagttattgattttaaccttgaattattattgcttgatgttaggtgcttatttcgccattccgcaataatcttaaaaagttcccttgcatttacattttgaaacatctatagcgataaatgaaacatcttaaaagttttagtatcatattcgtgttggattattctgcatttttggggagaatggacttgccgactgattaatgagggttaatcagtatgcagtggcataaaaaagcaaataaaggcatataacagatcgatcttaaacatccacaggaggatgggatccaaaataaggaggaaaaaaaaatgactagcaccggctatacgagcatcaacgggaagcatttttatttcaataccgacggcattatgcagatcggggtgttcaaagggcccaacggtttcgaatactttgcgccggccaacacggatgcgaataacatcgaaggtcaagccatcctctaccagaacaaattcctgaccctcaatggcaagaaatattacttcgggtccgacagcaaggctgtcacgggtctgcgcacgattgatgggaaaaagtattacttcaacaccaatactgccgtggcggtcaccggatggcaaacgatcaacggcaagaaatactacttcaataccaacacgtccattgcctcgaccgggtatacgatcatttccggcaaacacttctacttcaacaccgacgggatcatgcaaatcggtgtgtttaaagggcccgatggcttcgagtactttgccccggcgaatacggacgccaataacattgaaggtcaggcaattcggtatcagaatcgttttctctatctgcatgacaacatctactatttcggtaataacagcaaggcggccaccgggtgggtcacgattgatggcaaccggtattacttcgagcccaatacggcgatgggggcgaatggttataaaacgatcgacaacaagaatttctactttcgcaacgggctcccgcagattggcgtgttcaaagggtccaacggctttgagtacttcgcccccgcgaatacggatgccaacaatatcgagggccaagcgattcggtatcaaaaccgcttcctccacctgctcgggaaaatctattacttcggcaataactcgaaagccgtcacgggttggcaaacgattaatggcaaagtgtattacttcatgccggatactgcaatggcagccgctggtggattattcgaaattgacggcgtcatctatttctttggcgtggatggggtcaaagccccggggatctatggctaatgacctagctgataacctagcccgcctaatgagcgggcttttttttctcggcctagcgctggagctgcttcgaagttcctatactttctagagaataggaacttcgaactgcaggtcgacggatccactagtgtcgataacccttcctgtgttttcatgaacaggtaaaagtgaatttaaccctctgtttttgcagagggtttttatttatgtgcatagatgcattttctgtgtagtgcacagcttctggcggcaaagcactgcatcgacacaatagtgggtttcactggcagcacacaatcaaatctgacagtcggcttcgagcgaggtgcggacattggtagcttcaacaacatgactggcattgaggtgtattaatcaacgggaagcaggtcagtttactccgccagcccgacttttacgaaagggctaccatgactacgcgattttttgattagcttgccaacgtataatcctctgatttctggtgatgcgattcgtccaacaaattctgaacggttggtttcgggggggggatgaccaattcccgggtaaagtattgctgagagcctgccttcaaccagcactgtatctcgtaaacttccatcaccaaaccgccgtaggtggcgtatgcaaattgtaggttttcatcttttggtacttttgcccagacgccacgcgtagcttcatataatgcaagtgcactcatgccagacttgtaggtgctgtttagcaaaaaagcgagcccggcatgttcaggtgcgatttccgtctcttgcttaagaagaagatgattgagctcatccagcgtgattcgccccataagggagctgcttcctcgtactttgttggtcagttctccaacacccaagagatcaatacatgttgcttcaacaagcttcgcggttgcctcatccatgccatg

SEQ ID NO: 32 - DNA, 3229 bp, Artificial Sequence
  5htrA-PompC-14CBDA-FRT-3htrA gene cassette
gtgtcgccgatcttgaagacgcggtagagaaaagaatctttagcgttgagcagctttatcaccatttatatcacgcgtggggccaccatgagaaggattcgctgtttgagctggtggtaggaaatgcgtgggaaaaatcacgcgccaatacattaagccgcagtaccgaagatcagttttttatgtatttacgggtaaatacattaaataaactggtgccctatgccgctcagcgttttattgataatttgccgcagatttttgccggtaccttcaatcaggcgttactggaagatgccagcggttttagccgcctgcttgaactctataagaatgtggcggttgaacatgtgtttagccatccggatgtagaacagcttgaactacagggataccgggtgatcagcgggttattagatatctatcagccgctattaagcttgtcgcttaacgactttcgcgagctggtggaaaaagaacggttgaaacgcttccctatagaatcgcgcttatttcagaaactttctacgcgccatcgtttggcctacgtggaagtcgtcagtaaattacccacggattcggcggagtacccggtactggaatattattatcgctgtcggttgattcaggattatatcagcgggatgactgacctttacgcatgggatgaatatcggcgtttgatggcggtcgaacagtaaatggacttttgtaaagatggacaataaatttttactttttccagaaactttattccggaacttcgcgttataaaatgaatctgacgtacacagcaattttgcgttacctgttaatcgcaattcgtcaattctgtggtagcacagaataatgaaaagtgtgtaaagaagggtaaaaaaaaccgaatgcgaggcatccggttgaaataggggtaaacagacattcagaaatgaatgacggtaataaataaagttaatgatgatagcgggagttattctagttgcgagtgaaggttttgttttgacattcagtgctgtcaaatacttaagaataagttattgattttaaccttgaattattattgcttgatgttaggtgcttatttcgccattccgcaataatcttaaaaagttcccttgcatttacattttgaaacatctatagcgataaatgaaacatcttaaaagttttagtatcatattcgtgttggattattctgcatttttggggagaatggacttgccgactgattaatgagggttaatcagtatgcagtggcataaaaaagcaaataaaggcatataacagatcgatcttaaacatccacaggaggatgggatccaaaataaggaggaaaaaaaaatgactagcaccggctatacgagcatcaacgggaagcatttttatttcaataccgacggcattatgcagatcggggtgttcaaagggcccaacggtttcgaatactttgcgccggccaacacggatgcgaataacatcgaaggtcaagccatcctctaccagaacaaattcctgaccctcaatggcaagaaatattacttcgggtccgacagcaaggctgtcacgggtctgcgcacgattgatgggaaaaagtattacttcaacaccaatactgccgtggcggtcaccggatggcaaacgatcaacggcaagaaatactacttcaataccaacacgtccattgcctcgaccgggtatacgatcatttccggcaaacacttctacttcaacaccgacgggatcatgcaaatcggtgtgtttaaagggcccgatggcttcgagtactttgccccggcgaatacggacgccaataacattgaaggtcaggcaattcggtatcagaatcgttttctctatctgcatgacaacatctactatttcggtaataacagcaaggcggccaccgggtgggtcacgattgatggcaaccggtattacttcgagcccaatacggcgatgggggcgaatggttataaaacgatcgacaacaagaatttctactttcgcaacgggctcccgcagattggcgtgttcaaagggtccaacggctttgagtacttcgcccccgcgaatacggatgccaacaatatcgagggccaagcgattcggtatcaaaaccgcttcctccacctgctcgggaaaatctattacttcggcaataactcgaaagccgtcacgggttggcaaacgattaatggcaaagtgtattacttcatgccggatactgcaatggcagccgctggtggattattcgaaattgacggcgtcatctatttctttggcgtggatggggtcaaagccccggggatctatggctaatgacctagctgataacctagcccgcctaatgagcgggcttttttttctcggcctagcgctggagctgcttcgaagttcctatactttctagagaataggaacttcgaactgcaggtcgacggatccactagtctgcgtaagattctcgacagcaagccgtcggtgctggcgctgaatattcagcgtggtgatagttctatttatttgctgatgcagtaatcacctttgtcccccttccaccacggaagggggcaacacttttctgtgaaactccccacaactccatacttctttgcaccgttttgtgcatttgcacaatgtcgaggcctgtcatcttccttatgcttgtgctctgctcacaggagggatttatggctggctggcatcttgataccaaaatggcgcaggatatcgtggcgcgcactatgcgcatcatcgataccaatatcaacgtaatggatgcccgcgggcgtattatcggcagcggcgatcgggaacgtattggtgaattgcacgaaggcgcgttgttagtgctgtcacagggccgggttgtggatatcgacaacgccgtggcgcgacacctgcacggggtgcgtcaggggattaatcttcccttacgccttgagggcgaaattgttggcgtgatcggtctcaccggcgaaccagagcatctgcgtaaatatggcgaactggtgtgtatgactgccgaaatgatgctggaacagtcgcggttaatgcaccttttggcgcaggatagccgtttgcgtgaagagctggtgatgaacctgattcaggccgaagaaaatacgccggcgctggtggaatgggcacagcgtttagggatcgatttgaaccagccgcgtgtggcggcggtggtggaagtcgacagcggccagcttggcgtcgatag

SEQ ID NO: 33 - DNA, 2982 bp, Artificial Sequence
  5rpoS-PompC-14CBDA-FRT-3rpoS gene cassette
atgcagcacagcaaggagttgtgaccaggtctgcacaaaattccaccgttgcagttgcgtctcaaccaacaattacgtattctgagggctcaggtgaacaaagtgctaacaaaatgttgccaaacaacaagcctgctgggacggttgtcacagcgcctgtaacggcaccaacggtaagcacgaccgaaccaaatgcaagcagtacgtcaaccagcgcgccgatttccgcatggcgctggccgacggatggcaaagtgatcgaaaactttggcgcttccgaagggggcaataaagggatcgacattgcaggcagtaagggacaggctatcgtcgcaaccgctgatgggcgcgtcgtatatgccggtaacgcactgcgtggttacggtaatcttattatcatcaaacataacgatgattacctgagtgcctacgcccataatgatacgatgctggtccgggaacaacaggaagttaaggcggggcaaaaaatcgctactatgggtagcaccggcaccagctctacacgcttgcattttgaaattcgttacaaggggaaatccgtaaacccgctgcgttatttaccgcagcgataaagcggcggaaccaggctttgacttgctagttccgtcaagggatcacgggtcaattcgtcaattctgtggtagcacagaataatgaaaagtgtgtaaagaagggtaaaaaaaaccgaatgcgaggcatccggttgaaataggggtaaacagacattcagaaatgaatgacggtaataaataaagttaatgatgatagcgggagttattctagttgcgagtgaaggttttgttttgacattcagtgctgtcaaatacttaagaataagttattgattttaaccttgaattattattgcttgatgttaggtgcttatttcgccattccgcaataatcttaaaaagttcccttgcatttacattttgaaacatctatagcgataaatgaaacatcttaaaagttttagtatcatattcgtgttggattattctgcatttttggggagaatggacttgccgactgattaatgagggttaatcagtatgcagtggcataaaaaagcaaataaaggcatataacagatcgatcttaaacatccacaggaggatgggatccaaaataaggaggaaaaaaaaatgactagcaccggctatacgagcatcaacgggaagcatttttatttcaataccgacggcattatgcagatcggggtgttcaaagggcccaacggtttcgaatactttgcgccggccaacacggatgcgaataacatcgaaggtcaagccatcctctaccagaacaaattcctgaccctcaatggcaagaaatattacttcgggtccgacagcaaggctgtcacgggtctgcgcacgattgatgggaaaaagtattacttcaacaccaatactgccgtggcggtcaccggatggcaaacgatcaacggcaagaaatactacttcaataccaacacgtccattgcctcgaccgggtatacgatcatttccggcaaacacttctacttcaacaccgacgggatcatgcaaatcggtgtgtttaaagggcccgatggcttcgagtactttgccccggcgaatacggacgccaataacattgaaggtcaggcaattcggtatcagaatcgttttctctatctgcatgacaacatctactatttcggtaataacagcaaggcggccaccgggtgggtcacgattgatggcaaccggtattacttcgagcccaatacggcgatgggggcgaatggttataaaacgatcgacaacaagaatttctactttcgcaacgggctcccgcagattggcgtgttcaaagggtccaacggctttgagtacttcgcccccgcgaatacggatgccaacaatatcgagggccaagcgattcggtatcaaaaccgcttcctccacctgctcgggaaaatctattacttcggcaataactcgaaagccgtcacgggttggcaaacgattaatggcaaagtgtattacttcatgccggatactgcaatggcagccgctggtggattattcgaaattgacggcgtcatctatttctttggcgtggatggggtcaaagccccggggatctatggctaatgacctagctgataacctagcccgcctaatgagcgggcttttttttctcggcctagcgacgaattgcctagcgctggagctgcttcgaagttcctatactttctagagaataggaacttcgaactgcaggtcgacggatccggttcggtatcgcgccaggtatacagacaatgctgacactgatataccgtccagactccttttaccggcgaagtcgccatgagttcaatatgtgcatcggcacagcgtggacaaatcatcggttactccttatttacggttggccagcatggcggtcagcttttcagcccaggctttagtttccggtaaatccacaaccggctggctatagtgaccacggttatctggcgcaaccggcgtggtagcgtcaatgatcagtttgtcggtaatccccgccgggcttgaacccgggtccagttccaggacggacatattcggtagctgtaccagatcgcctgccggattcactttcgacgacaacgcccacatcacctgtggcagattaaatggatcgacatcttcatcaaccatgatcaccatcttcacatatcccagaccgtgcggcgtcgtcatcgcgcgcaggcccaccgcacgggcaaagccgccgtagcgttttttggtcgagatgatggccagcaagccgtgggtgtacatagcgtttaccgcctgcacttccggaaattcggctttcagctgttgatacagtggcacacaggtcgccggccccatcaggtagtcgatttccgtccacggcatccccaaatagagcgattcaaaaatgggtttgctgtggtaagagaccttatcgatacgcacc

SEQ ID NO: 34 - protein, 325 aa, Clostridium difficile
MTSTGYTSINGKHFYFNTDGIMQIGVFKGPNGFEYFAPANTDANNIEGQAILYQNKFLTLNGKKYYFGSDSKAVTGLRTIDGKKYYFNTNTAVAVTGWQTINGKKYYFNTNTSIASTGYTIISGKHFYFNTDGIMQIGVFKGPDGFEYFAPANTDANNIEGQAIRYQNRFLYLHDNIYYFGNNSKAATGWVTIDGNRYYFEPNTAMGANGYKTIDNKNFYFRNGLPQIGVFKGSNGFEYFAPANTDANNIEGQAIRYQNRFLHLLGKIYYFGNNSKAVTGWQTINGKVYYFMPDTAMAAAGGLFEIDGVIYFFGVDGVKAPGIYG

SEQ ID NO: 35 - DNA, 1542 bp, Artificial Sequence
  ssb region of chromosomal deletion
ttcggcggatcggagagatcgcagacttcgccgtcaatacgggcgcgaatgtaaccctggcttgccagattttccagcgttttggtgtgttcgcctttacgctctttaataatcggcgccagcagcatcaggcgtttgccttccggctgcgacagcacgttatcgaccatctggctaacggtttgcgccgccagcggcacgtcatggtccggacaacgcggctcgcccacgcgggcaaacagcaggcgcaggtagtcgtggatctcggtaatagtacccaccgtagagcgcgggttgtgcgatgtcgatttctgttcaattgagatcgcgggcgatagcccctcaatatggtcgacatccggtttttccatgagcgacaaaaactgccgcgcgtaagcggagagcgattcaacgtaacgacgctgcccttcggcatacagagtgtcgaaagccagtgaggatttgcctgaacccgaaagcccggtcacgacaatcagtttgtcgcgggggatgacgaggttaatatttttgagattatgggtgcgggcgccccgaacttcgatcttatccattcacctttcccggtagagactcggatgcctggtttgtttgaaggacaaacggcagaaacggctaattatgacacaatttaacctgtttgaatatacagtagctagcgtgtaggctggagctgcttcgaagttcctatactttctagagaataggaacttcggaataggaactaaggaggatattcatatgcattttcgctatagttctcgtctgctgaaatgcctggtgtaaaccaggcattttattacctggtattattgtcttagtatccctttcaaaaaagagaagcgcatatctcacggaatgacttacggaaaaatgtcgcttatcgcctctggccgactcgcctcggcacatcattatccagccgaagttcataaatgtactgcaataacccggattgtcttaaatatgaaagagaaatctcatctgcaaaatatataatttatagccattttttgacaacaaaaagatattataaaataacggtagagaatggtcggtattatcaatagttaattaaatgcttgctttagcttgtgatgagctcaaatatgatatgtgtatcttgctttatttttaattgctgaagataaaattgttacttatagctggctttatataaaaaatggttttatttgtgtatttttttacacaattctgattttttactccccacttattatattttcaatgatttaagttatattgaagtccctatgaccctatgttttaattgtgaaaattcattttatcctctggaggcaaatttattaaatacgtatggttataacgcgtattaaaaagaaatatgtccttaaaatgatttagagtttcaatgattagctaacaaatctatttatcggcgggtggttttaatttgctgatgactattttttatttatgagctgagagcttatgcgatacctattattggggaagatatagttagtgcaataattgatgtct

SEQ ID NO: 36 - DNA, 8045 bp, Artificial Sequence
  PompC-clyA-cbd/b cassette
gaattctgtggtagcacagaataatgaaaagtgtgtaaagaagggtaaaaaaaaccgaatgcgaggcatccggttgaaataggggtaaacagacattcagaaatgaatgacggtaataaataaagttaatgatgatagcgggagttattctagttgcgagtgaaggttttgttttgacattcagtgctgtcaaatacttaagaataagttattgattttaaccttgaattattattgcttgatgttaggtgcttatttcgccattccgcaataatcttaaaaagttcccttgcatttacattttgaaacatctatagcgataaatgaaacatcttaaaagttttagtatcatattcgtgttggattattctgcatttttggggagaatggacttgccgactgattaatgagggttaatcagtatgcagtggcataaaaaagcaaataaaggcatataacagatcgatcttaaacatccacaggaggatgggatccaaaataaggaggaaaaaaaaatgactagtatttttgcagaacaaactgtagaggtagttaaaagcgcgatcgaaaccgcagatggggcattagatctttataacaaatacctcgaccaggtcatcccctggaagacctttgatgaaaccataaaagagttaagccgttttaaacaggagtactcgcaggaagcttctgttttagttggtgatattaaagttttgcttatggacagccaggacaagtattttgaagcgacacaaactgtttatgaatggtgtggtgtcgtgacgcaattactctcagcgtatattttactatttgatgaatataatgagaaaaaagcatcagcccagaaagacattctcattaggatattagatgatggtgtcaagaaactgaatgaagcgcaaaaatctctcctgacaagttcacaaagtttcaacaacgcttccggaaaactgctggcattagatagccagttaactaatgatttttcggaaaaaagtagttatttccagtcacaggtggatagaattcgtaaggaagcttatgccggtgctgcagccggcatagtcgccggtccgtttggattaattatttcctattctattgctgcgggcgtgattgaagggaaattgattccagaattgaataacaggctaaaaacagtgcaaaatttctttactagcttatcagctacagtgaaacaagcgaataaagatatcgatgcggcaaaattgaaattagccactgaaatagcagcaattggggagataaaaacggaaaccgaaacaaccagattctacgttgattatgatgatttaatgctttctttattaaaaggagctgcaaagaaaatgattaacacctgtaatgaataccaacaacgtcatggtaagaagacgcttttcgaggttcctgacgtcgctagcggcctgatctatattaacgattcactgtactatttcaagccgcccgtcaataacctcatcaccgggtttgtgacggtcggcgacgataaatactacttcaatccgatcaacggcggagccgcgagcattggggagaccatcattgatgacaagaattattacttcaaccagagtggcgtgctgcagacgggggtcttcagtaccgaggacggctttaaatacttcgcccccgcgaatacgctcgatgagaacctggaaggggaggcgattgactttaccggcaagctgatcattgacgagaacatctactatttcgatgacaattaccgcggggccgtggaatggaaggagctcgatggcgagatgcactattttagcccggagacggggaaagctttcaaaggcctgaatcaaattggggactacaagtattacttcaactctgacggtgtgatgcagaaggggttcgtgagtatcaatgacaacaagcattatttcgacgattctggcgtcatgaaagtggggtacaccgagatcgatggcaagcacttctactttgccgagaatggtgagatgcaaatcggcgtgttcaatacggaagacgggtttaagtatttcgcgcatcataacgaggatctcggcaatgaagagggcgaagagatctcatattccggaatcctcaacttcaataacaagatttactactttgatgactcatttaccgccgtggtcggctggaaggacctcgaggatgggtcaaagtactatttcgacgaggatacggcggaggcctacatcggcctgtcattaatcaacgacggccagtattactttaatgatgacggcatcatgcaggtcgggtttgtcaccatcaacgataaagtcttctacttctctgactctggcattatcgagagcggggtgcagaacatcgacgataactatttctacatcgatgacaatggcattgtccagatcggcgtgttcgatacgtcagacggttataagtattttgcgcccgccaacaccgtcaacgataatatctacggtcaagctgttgaatatagtggtttggtccgtgtcggtgaagacgtgtactatttcggcgagacgtacacaattgagacgggctggatctatgatatggagaacgagagtgacaagtactatttcaatcctgagaccaagaaagcatgcaaggggatcaacctgatcgatgacatcaagtactatttcgacgagaagggcattatgcgcacggggcttatctcatttgagaataacaattattacttcaatgagaacggggaaatgcagtttgggtacatcaatattgaggacaagatgttctattttggcgaggatggcgtcatgcagatcggggtgttcaacaccccagatggtttcaagtatttcgcgcatcagaatacgctggatgagaacttcgagggcgaatcaatcaactataccgggtggctggacctcgatgagaagcgctactatttcacggacgaatacattgcggccaccggctcagtcatcattgatggcgaggaatactatttcgaccctgatacggcgcagctggtgatcagtgagtaatgacctagctgataacctagcccgcctaatgagcgggcttttttttctcggcctaggtttcacctgttctattaggtgttacatgctgttcatctgttacattgtcgatctgttcatggtgaacagctttaaatgcaccaaaaactcgtaaaagctctgatgtatctatcttttttacaccgttttcatctgtgcatatggacagttttccctttgatatctaacggtgaacagttgttctacttttgtttgttagtcttgatgcttcactgatagatacaagagccataagaacctcagatccttccgtatttagccagtatgttctctagtgtggttcgttgtttttgcgtgagccatgagaacgaaccattgagatcatgcttactttgcatgtcactcaaaaattttgcctcaaaactggtgagctgaatttttgcagttaaagcatcgtgtagtgtttttcttagtccgttacgtaggtaggaatctgatgtaatggttgttggtattttgtcaccattcatttttatctggttgttctcaagttcggttacgagatccatttgtctatctagttcaacttggaaaatcaacgtatcagtcgggcggcctcgcttatcaaccaccaatttcatattgctgtaagtgtttaaatctttacttattggtttcaaaacccattggttaagccttttaaactcatggtagttattttcaagcattaacatgaacttaaattcatcaaggctaatctctatatttgccttgtgagttttcttttgtgttagttcttttaataaccactcataaatcctcatagagtatttgttttcaaaagacttaacatgttccagattatattttatgaatttttttaactggaaaagataaggcaatatctcttcactaaaaactaattctaatttttcgcttgagaacttggcatagtttgtccactggaaaatctcaaagcctttaaccaaaggattcctgatttccacagttctcgtcatcagctctctggttgctttagctaatacaccataagcattttccctactgatgttcatcatctgagcgtattggttataagtgaacgataccgtccgttctttccttgtagggttttcaatcgtggggttgagtagtgccacacagcataaaattagcttggtttcatgctccgttaagtcatagcgactaatcgctagttcatttgctttgaaaacaactaattcagacatacatctcaattggtctaggtgattttaatcactataccaattgagatgggctagtcaatgataattactagctagtccttttcctttgagttgtgggtatctgtaaattctgctagacctttgctggaaaacttgtaaattctgctagaccctctgtaaattccgctagacctttgtgtgttttttttgtttatattcaagtggttataatttatagaataaagaaagaataaaaaaagataaaaagaatagatcccagccctgtgtataactcactactttagtcagttccgcagtattacaaaaggatgtcgcaaacgctgtttgctcctctacaaaacagaccttaaaaccctaaaggcttaagtagcaccctcgcaagctcgggcaaatcgctgaatattccttttgtctccgaccatcaggcacctgagtcgctgtctttttcgtgacattcagttcgctgcgctcacggctctggcagtgaatgggggtaaatggcactacaggcgccttttatggattcatgcaaggaaactacccataatacaagaaaagcccgtcacgggcttctcagggcgttttatggcgggtctgctatgtggtgctatctgactttttgctgttcagcagttcctgccctctgattttccagtctgaccacttcggattatcccgtgacaggtcattcagactggctaatgcacccagtaaggcagcggtatcatcaacaggcttacccgtcttactgtcaaccggatctaaaacactaggcccaagagtttgtagaaacgcaaaaaggccatccgtcaggatggccttctgcttaatttgatgcctggcagtttatggcgggcgtcctgcccgccaccctccgggccgttgcttcgcaacgttcaaatccgctcccggcggatttgtcctactcaggagagcgttcaccgacaaacaacagataaaacgaaaggcccagtctttcgactgagcctttcgttttatttgatgcctggcagttccctactctcgcatggggagaccccacactaccatcggcgctacggcgtttcacttctgagttcggcatggggtcaggtgggaccaccgcgctactgccgccaggcaaattctgttttatcagaccgcttctgcgttctgatttaatctgtatcaggctgaaaatcttctctcatccgccaaaacagccaagctggatctaaaacactagctctagctattgttttaatgacaaatcagaacggaatgtcatcatcaaagtccatcggcggctcgttagacggcgctgccggagcggactgctgcgggcgagactgcgcgccgccgctgaactgattgccaccctgcggctgctgaggctgaccccaaccgccctgcggctgaccaccaccgatattgccacctgccggagcgccaccaccctgacgaccacccagcatctgcatggtgccgccaacgttcaccacgacttctgtggtgtagcgatcctgaccggattgatcggtccatttacgggtacgcagctgaccttcgatataaacctgagaacctttacgcagatattcgctcgccacttctgccagtttgccgaacagcacaacgcggtgccattcagtctgttctttcatctcgccggtcgctttatcacgccaggattcggaagtagccagcgtaatgttggcaactgcgccaccatttggcatgtagcgtacttccgggtcctgacccagattaccaacgagaataaccttgtttacgcctctgctggccatgttcgtgtctcctgaaaaaaatcgttctgaataagtgtaaacgcgcgattgtaccattaccaatagcgcttttactatgttgtgacctcggttccgggaaacaaacctggccagacattgttacacaacactccggataatgcattccaatactgtatattcattcaggtcaatcatatgaagggcgaattctgcagatatccatcacactggcggccgccagtgtgatggatatctgcagaattcgcccttgagaagttcctattctatatatagtataggaacttctctagaacttttgttacccgccaaacaaaacccaaaaacaacccatacccaacccaataaaacaccaaaacaagacaaataatcattgattgatggttgaaatggggtaaacttgacaaacaaacccacttaaaacccaaaacatacccaaacacacaccaaaaaaacaccataaggagttttataaatgttggtattcattgatgacggttcaacaaacatcaaactacagtggcaggaaagcgacggaacaattaaacagcacattagcccgaacagcttcaaacgcgagtgggcagtctcttttggtgataaaaaggtctttaactacacactgaacggcgaacagtattcatttgatccaatcagcccggatgctgtagtcacaaccaatatcgcatggcaatacagcgacgttaatgtcgttgcagtgcatcacgccttactgaccagtggtctgccggtaagcgaagtggatattgtttgcacacttcctctgacagagtattacgacagaaataaccaacccaatacggaaaatattgagcgtaagaaagcaaacttccggaaaaaaattacattaaatggcggggatacattcacaataaaagatgtaaaagtcatgcctgaatctataccggcaggttatgaagttctacaagaactggatgagttagattctttattaattatagatctcgggggcaccacattagatatttctcaggtaatggggaaattatcggggatcagtaaaatatacggagactcatctcttggtgtctctctggttacatctgcagtaaaagatgccctttctcttgcgagaacaaaaggaagtagctatcttgctgacgatataatcattcacagaaaagataataactatctgaagcaacgaattaatgatgagaacaaaatatcaatagtcaccgaagcaatgaatgaagcacttcgtaaacttgagcaacgtgtattaaatacgctcaatgaattttctggttatactcatgttatggttataggcggtggcgcagaattaatatgcgatgcagtaaaaaaacacacacagattcgtgatgaacgttttttcaaaaccaataactctcaatatgatttagttaacggtatgtatctcataggtaattaatgatggacaagcgcagaaccattgccttcaaactaaatccagatgtaaatcaaacagataaaattgtttgtgatacactggacagtatcccgcaaggggaacgaagccgccttaaccgggccgcactgacggcaggtctggccttatacagacaagatccccggacccctttccttttatgtgagctgctgacgaaagaaaccacattttcagatatcgtgaatatattgagatcgctatttccaaaagagatggccgattttaattcttcaatagtcactcaatcctcttcacaacaagagcaaaaaagtgatgaagagaccaaaaaaaatgcgatgaagctaataaattaattcaattattattgagttccctttatccactatcaggctggataaagggaactcaatcaagttattttcttaccagtcattacataatcgttattatgaaataatcgtttgcactgtctctgttattcaggcaatttcaataaaggcacttgctcacgctctgtcattttctgaaactcttcatgctg

SEQ ID NO: 37 - protein, 838 aa, Artificial Sequence
  Amino acid sequence of ClyA-CBD/B
MTSIFAEQTVEVVKSAIETADGALDLYNKYLDQVIPWKTFDETIKELSRFKQEYSQEASVLVGDIKVLLMDSQDKYFEATQTVYEWCGVVTQLLSAYILLFDEYNEKKASAQKDILIRILDDGVKKLNEAQKSLLTSSQSFNNASGKLLALDSQLTNDFSEKSSYFQSQVDRIRKEAYAGAAAGIVAGPFGLIISYSIAAGVIEGKLIPELNNRLKTVQNFFTSLSATVKQANKDIDAAKLKLATEIAAIGEIKTETETTRFYVDYDDLMLSLLKGAAKKMINTCNEYQQRHGKKTLFEVPDVASGLIYINDSLYYFKPPVNNLITGFVTVGDDKYYFNPINGGAASIGETIIDDKNYYFNQSGVLQTGVFSTEDGFKYFAPANTLDENLEGEAIDFTGKLIIDENIYYFDDNYRGAVEWKELDGEMHYFSPETGKAFKGLNQIGDYKYYFNSDGVMQKGFVSINDNKHYFDDSGVMKVGYTEIDGKHFYFAENGEMQIGVFNTEDGFKYFAHHNEDLGNEEGEEISYSGILNFNNKIYYFDDSFTAVVGWKDLEDGSKYYFDEDTAEAYIGLSLINDGQYYFNDDGIMQVGFVTINDKVFYFSDSGIIESGVQNIDDNYFYIDDNGIVQIGVFDTSDGYKYFAPANTVNDNIYGQAVEYSGLVRVGEDVYYFGETYTIETGWIYDMENESDKYYFNPETKKACKGINLIDDIKYYFDEKGIMRTGLISFENNNYYFNENGEMQFGYINIEDKMFYFGEDGVMQIGVFNTPDGFKYFAHQNTLDENFEGESINYTGWLDLDEKRYYFTDEYIAATGSVIIDGEEYYFDPDTAQLVISE

SEQ ID NO: 38 - protein, 305 aa, Salmonella typhi
MTSIFAEQTVEVVKSAIETADGALDLYNKYLDQVIPWKTFDETIKELSRFKQEYSQEASVLVGDIKVLLMDSQDKYFEATQTVYEWCGVVTQLLSAYILLFDEYNEKKASAQKDILIRILDDGVKKLNEAQKSLLTSSQSFNNASGKLLALDSQLTNDFSEKSSYFQSQVDRIRKEAYAGAAAGIVAGPFGLIISYSIAAGVIEGKLIPELNNRLKTVQNFFTSLSATVKQANKDIDAAKLKLATEIAAIGEIKTETETTRFYVDYDDLMLSLLKGAAKKMINTCNEYQQRHGKKTLFEVPDVAS

SEQ ID NO: 39 - DNA, 921 bp, Salmonella typhi
atgactagtatttttgcagaacaaactgtagaggtagttaaaagcgcgatcgaaaccgcagatggggcattagatctttataacaaatacctcgaccaggtcatcccctggaagacctttgatgaaaccataaaagagttaagccgttttaaacaggagtactcgcaggaagcttctgttttagttggtgatattaaagttttgcttatggacagccaggacaagtattttgaagcgacacaaactgtttatgaatggtgtggtgtcgtgacgcaattactctcagcgtatattttactatttgatgaatataatgagaaaaaagcatcagcccagaaagacattctcattaggatattagatgatggtgtcaagaaactgaatgaagcgcaaaaatctctcctgacaagttcacaaagtttcaacaacgcttccggaaaactgctggcattagatagccagttaactaatgatttttcggaaaaaagtagttatttccagtcacaggtggatagaattcgtaaggaagcttatgccggtgctgcagccggcatagtcgccggtccgtttggattaattatttcctattctattgctgcgggcgtgattgaagggaaattgattccagaattgaataacaggctaaaaacagtgcaaaatttctttactagcttatcagctacagtgaaacaagcgaataaagatatcgatgcggcaaaattgaaattagccactgaaatagcagcaattggggagataaaaacggaaaccgaaacaaccagattctacgttgattatgatgatttaatgctttctttattaaaaggagctgcaaagaaaatgattaacacctgtaatgaataccaacaacgtcatggtaagaagacgcttttcgaggttcctgacgtcgctagctgataa

SEQ ID NO: 40 - DNA, 909 bp, Artificial Sequence
  chemically-synthesized codon-optimized S. Typhi clyA polynucleotide sequence
atgactagtatttttgcggaacagaccgtggaagtggttaaaagcgcgatcgaaaccgcggatggcgcgttagatctttataacaaatatctggatcaggtgattccgtggaaaacctttgatgaaaccattaaagaactgagccgttttaaacaggaatatagccaggaagcgagcgtgctggtgggcgatattaaagtgctgctgatggatagccaggataaatattttgaagcgacccagaccgtgtatgaatggtgcggcgtggttacccagctgctgagcgcgtatatcctgctgtttgatgaatataacgaaaagaaagcgagcgctcagaaagatattctgattcgtattctggatgacggcgtgaaaaaactgaacgaagcgcagaaaagcctgctgaccagcagccagagctttaacaatgcgtccggaaaactgctggcgctggatagccagctgaccaacgattttagcgaaaaaagcagctattttcagagccaggtggatagaattcgtaaagaagcctatgccggcgctgcagccggcattgtggctggtccgtttggcctgattatcagctatagcattgccgcgggcgttattgaaggcaaactgattccggaactgaataaccgtctgaaaaccgttcagaatttctttacaagcttaagcgcgaccgtgaaacaggcgaacaaagatatcgatgcggcaaaactgaaactggcgaccgaaattgcggctattggcgaaattaaaaccgaaaccgaaaccacccgtttttatgtggattatgatgacctgatgctgagcctgctgaaaggcgcggcaaagaaaatgattaacacctgcaacgaatatcagcagcgtcatggcaagaaaaccctgtttgaagtgccggatgtg

SEQ ID NO: 41 - DNA, 1102 bp, Salmonella typhi
ggaggtaataggtaagaatactttataaaacaggtacttaattgcaatttatatatttaaagaggcaaatgattatgaccggaatatttgcagaacaaactgtagaggtagttaaaagcgcgatcgaaaccgcagatggggcattagatctttataacaaatacctcgaccaggtcatcccctggaagacctttgatgaaaccataaaagagttaagccgttttaaacaggagtactcgcaggaagcttctgttttagttggtgatattaaagttttgcttatggacagccaggacaagtattttgaagcgacacaaactgtttatgaatggtgtggtgtcgtgacgcaattactctcagcgtatattttactatttgatgaatataatgagaaaaaagcatcagcccagaaagacattctcattaggatattagatgatggtgtcaagaaactgaatgaagcgcaaaaatctctcctgacaagttcacaaagtttcaacaacgcttccggaaaactgctggcattagatagccagttaactaatgatttttcggaaaaaagtagttatttccagtcacaggtggatagaattcgtaaggaagcttatgccggtgctgcagccggcatagtcgccggtccgtttggattaattatttcctattctattgctgcgggcgtgattgaagggaaattgattccagaattgaataacaggctaaaaacagtgcaaaatttctttactagcttatcagctacagtgaaacaagcgaataaagatatcgatgcggcaaaattgaaattagccactgaaatagcagcaattggggagataaaaacggaaaccgaaacaaccagattctacgttgattatgatgatttaatgctttctttattaaaaggagctgcaaagaaaatgattaacacctgtaatgaataccaacaaagacacggtaagaagacgcttttcgaggttcctgacgtctgatacattttcattcgatctgtgtacttttaacgcccgatagcgtaaagaaaatgagagacggagaaaaagcgatattcaacagcccgataaacaagagtcgttaccgggctgacgag

SEQ ID NO: 42 - DNA, 1102 bp, Salmonella paratyphi
ggaggcaataggtaggaataagttataaaacaatagcttaattgcaatttatatatttaaagaggcaaatgattatgactggaatatttgcagaacaaactgtagaggtagttaaaagcgcgatcgaaaccgcagatggggcattagatttttataacaaatacctcgaccaggttatcccctggaagacctttgatgaaaccataaaagagttaagccgttttaaacaggagtactcgcaggaagcttctgttttagttggtgatattaaagttttgcttatggacagccaggataagtattttgaagcgacacaaactgtttatgaatggtgtggtgtcgtgacgcaattactctcagcgtatattttactatttgatgaatataatgagaaaaaagcatcagcgcagaaagacattctcatcaggatattagatgatggcgtcaataaactgaatgaagcgcaaaaatctctcctgggaagttcacaaagtttcaacaacgcttcaggaaaactgctggcattagatagccagttaactaatgatttctcggaaaaaagtagttatttccagtcacaggtggatagaattcgtaaggaagcttatgccggtgctgcagcaggcatagtcgccggtccgtttggattaattatttcctattctattgctgcgggcgtgattgaagggaaattgattccagaattgaatgacaggctaaaagcagtgcaaaatttctttactagcttatcagtcacagtgaaacaagcgaataaagatatcgatgcggcaaaattgaaattagccactgaaatagcagcaattggggagataaaaacggaaaccgaaacaaccagattctacgttgattatgatgatttaatgctttctttactaaaaggagctgcaaagaaaatgattaacacctgtaatgaataccaacaaaggcacggtaagaagacgcttctcgaggttcctgacatctgatacattttcattcgctctgtttacttttaacgcccgatagcgtgaagaaaatgagagacggagaaaaagcgatattcaacagcccgataaacaagagtcgttaccgggctggcgag

SEQ ID NO: 43 - DNA, 904 bp, Shigella flexneri
atgactgaaatcgttgcagataaaacggtagaagtagttaaaaacgcaatcgaaaccgcagatggagcattagatctttataataaatatctcgatcaggtcatcccctggcagacctttgatgaaaccataaaagagttaagtcgctttaaacaggagtattcacaggcagcctccgttttagtcggcgatattaaaaccttacttatggatagccaggataagtattttgaagcaacccaaacagtgtatgaatggtgtggtgttgcgacgcaattgctcgcagcgtatattttgctatttgatgagtacaatgagaagaaagcatccgcccctcattaaggtactggatgacggcatcacgaagctgaatgaagcgcaaaattccctgctggtaagctcacaaagtttcaacaacgcttccgggaaactgctggcgttagatagccagttaaccaatgatttttcagaaaaaagcagctatttccagtcacaggtagataaaatcaggaaggaagcgtatgccggtgccgcagccggtgtcgtcgccggtccatttggtttaatcatttcctattctattgctgcgggcgtagttgaagggaaactgattccagaattgaagaacaagttaaaatctgtgcagagtttctttaccaccctgtctaacacggttaaacaagcgaataaagatatcgatgccgccaaattgaaattaaccaccgaaatagccgccatcggggagataaaaacggaaactgaaaccaccagattctatgttgattatgatgatttaatgctttctttgctaaaagcagcggccaaaaaaatgattaacacctgtaatgagtatcagaaaagacacggtaaaaagacactctttgaggtacctgaagtctgataa

SEQ ID NO: 44 - DNA, 1080 bp, Escherichia coli
agaaataaagacattgacgcatcccgcccggctaactatgaattagatgaagtaaaatttattaatagttgtaaaacaggagtttcattacaatttatatatttaaagaggcgaatgattatgactgaaatcgttgcagataaaacggtagaagtagttaaaaacgcaatcgaaaccgcagatggagcattagatctttataataaatatctcgatcaggtcatcccctggcagacctttgatgaaaccataaaagagttaagtcgctttaaacaggagtattcacaggcagcctccgttttagtcggcgatattaaaaccttacttatggatagccaggataagtattttgaagcaacccaaacagtgtatgaatggtgtggtgttgcgacgcaattgctcgcagcgtatattttgctatttgatgagtacaatgagaagaaagcatccgcccagaaagacattctcattaaggtactggatgacggcatcacgaagctgaatgaagcgcaaaaatccctgctggtaagctcacaaagtttcaacaacgcttccgggaaactgctggcgttagatagccagttaaccaatgatttttcagaaaaaagcagctatttccagtcacaggtagataaaatcaggaaggaagcatatgccggtgccgcagccggtgtcgtcgccggtccatttggattaatcatttcctattctattgctgcgggcgtagttgaaggaaaactgattccagaattgaagaacaagttaaaatctgtgcagaatttctttaccaccctgtctaacacggttaaacaagcgaataaagatatcgatgccgccaaattgaaattaaccaccgaaatagccgccatcggtgagataaaaacggaaactgaaacaaccagattctacgttgattatgatgatttaatgctttctttgctaaaagaagcggccaaaaaaatgattaacacctgtaatgagtatcagaaaagacacggtaaaaagacactctttgaggtacctgaagtctgataagcgattattctctccatgtactcaaggtataaggtttatcacatt